European Patent Application EP 4 667 014 A1, published December 24, 2025. Title: ASM 단백질 또는 이의 단편을 포함하는 퇴행성 신경질환 또는 우울증 예방 또는 치료용 조성물. Applicant: 경북대학교 산학협력단. The sequence listing filed with the application follows.

SEQUENCE LISTING (8 sequences)

SEQ ID NO: 1 - protein, 584 aa, synthetic construct
LALSDSRVLWAPAEAHPLSPQGHPARLHRIVPRLRDVFGWGNLTCPICKGLFTAINLGLKKEPNVARVGSVAIKLCNLLKIAPPAVCQSIVHLFEDDMVEVWRRSVLSPSEACGLLLGSTCGHWDIFSSWNISLPTVPKPPPKPPSPPAPGAPVSRILFLTDLHWDHDYLEGTDPDCADPLCCRRGSGLPPASRPGAGYWGEYSKCDLPLRTLESLLSGLGPAGPFDMVYWTGDIPAHDVWHQTRQDQLRALTTVTALVRKFLGPVPVYPAVGNHESTPVNSFPPPFIEGNHSSRWLYEAMAKAWEPWLPAEALRTLRIGGFYALSPYPGLRLISLNMNFCSRENFWLLINSTDPAGQLQWLVGELQAAEDRGDKVHIIGHIPPGHCLKSWSWNYYRIVARYENTLAAQFFGHTHVDEFEVFYDEETLSRPLAVAFLAPSATTYIGLNPGYRVYQIDGNYSGSSHVVLDHETYILNLTQANIPGAIPHWQLLYRARETYGLPNTLPTAWHNLVYRMRGDMQLFQTFWFLYHKGHPPSEPCGTPCRLATLCAQLSARADSPALCRHLMPDGSLPEAQSLWPRPLF

SEQ ID NO: 2 - protein, 85 aa, synthetic construct
GNLTCPICKGLFTAINLGLKKEPNVARVGSVAIKLCNLLKIAPPAVCQSIVHLFEDDMVEVWRRSVLSPSEACGLLLGSTCGHWD

SEQ ID NO: 3 - protein, 15 aa, synthetic construct
CGDIPAHDVWHQTRQ

SEQ ID NO: 4 - protein, 15 aa, synthetic construct
CEPWLPAEALRTLRI

SEQ ID NO: 5 - protein, 15 aa, synthetic construct
CLLYRARETYGLPNT

SEQ ID NO: 6 - protein, 15 aa, synthetic construct
CFIEGNHSSRWLYEA

SEQ ID NO: 7 - protein, 15 aa, synthetic construct
VEVWRRSVLSPSEAC

SEQ ID NO: 8 - protein, 14 aa, synthetic construct
CRRGSGLPPASRPG